European Patent Application EP 4 635 986 A1, published October 22, 2025. Title: ANTI-EC PEPTIDE MONOCLONAL ANTIBODY. Applicant: NATIONAL AND KAPODISTRIAN UNIVERSITY OF ATHENS. The sequence listing filed with the application follows.

SEQUENCE LISTING (4 sequences)

SEQ ID NO: 1 - protein, 24 aa, synthetic construct
YQPPSTNKNTKSQRRKGSTFEERK

SEQ ID NO: 2 - protein, 457 aa, synthetic construct
MGWTLVFLFLLSVTAGVHSEVQLQQSGAELVRSGASVKLSCAASGFNLKDYYIHWVKQRPEQGLEWIGWIDPENGDTEYAPKFQGRATMTADTSSNTAYLHLSSLTSEDTAVYYCFANDVDCWGQGTTLTVSSAKTTPPSVYPLAPGSAAQTNSMVTLGCLVKGYFPEPVTVTWNSGSLSSGVHTFPAVLESDLYTLSSSVTVPSSPRPSETVTCNVAHPASSTKVDKKIVPRDCGCKPCICTVPEVSSVFIFPPKPKDVLTITLTPKVTCVVVDISKDDPEVQFSWFVDDVEVHTAQTQPREEQFNSTFRSVSELPIMHQDWLNGKEFKCRVNSAAFPAPIEKTISKTKGRPKAPQVYTIPPPKEQMAKDKVSLTCMITDFFPEDITVEWQWNGQPAENYKNTQPIMNTNGSYFVYSKLNVQKSNWEAGNTFTCSVLHEGLHNHHTEKSLSHSPGK

SEQ ID NO: 3 - protein, 239 aa, synthetic construct
MVSSAQFLGLLLLCFQGTRCDVVMTQPPLSLPVSLGDQASISCRSSQSLVHSNGKTYLHWYLQKPGQSPKLLIYKLSNRFSGVPDRFSGSGSGTDFTLKISRVEAEDLGVYFCFQSTHIPYTFGGGSKLEIRRADAAPTVSIFPPSSEQLTSGGASVVCFLNNFYPKDINVKWKIDGSERQNGVLNSWTDQDSKDSTYSMSSTLTLTKDEYERHNSYTCEATHKTSTSPIVKSFNRNEC

SEQ ID NO: 4 - protein, 25 aa, synthetic construct
CSKNKTQSREGTKFSEKYRPNTRPQ